European Patent Application EP 4 349 867 A1, published April 10, 2024. Title: SPECIFIC BINDING PROTEIN TARGETING PD-L1 AND CD73. Applicant: Harbour BioMed (Shanghai) Co., Ltd. The sequence listing filed with the application follows.

SEQUENCE LISTING (157 sequences)

SEQ ID NO: 1 - protein, 25 aa, Artificial Sequence [sequence omitted]

SEQ ID NO: 2 - protein, 25 aa, Artificial Sequence
QVQLVESGGGVAQPGRSLSLSCAAS

SEQ ID NO: 3 - protein, 25 aa, Artificial Sequence
QVQLVESGGGVVQPGMSLRLSCAAS

SEQ ID NO: 4 - protein, 25 aa, Artificial Sequence
EVQLVESGGGVVQPGRSLRLSCAAS

SEQ ID NO: 5 - protein, 25 aa, Artificial Sequence
EVQLLESGGGVVQPGRSLRLSCAAS

SEQ ID NO: 6 - protein, 25 aa, Artificial Sequence
QVQLVESGGGVVQPGRSLRLSCAAS

SEQ ID NO: 7 - protein, 7 aa, Artificial Sequence
GFTFSDS

SEQ ID NO: 8 - protein, 7 aa, Artificial Sequence
GFTFSDY

SEQ ID NO: 9 - protein, 7 aa, Artificial Sequence
GFNFSNY

SEQ ID NO: 10 - protein, 7 aa, Artificial Sequence
GFTFSSY

SEQ ID NO: 11 - protein, 7 aa, Artificial Sequence
GFNFSSY

SEQ ID NO: 12 - protein, 7 aa, Artificial Sequence
GFTFYSY

SEQ ID NO: 13 - protein, 7 aa, Artificial Sequence
GFTFSNY

SEQ ID NO: 14 - protein, 7 aa, Artificial Sequence
GFDFSSY

SEQ ID NO: 15 - protein, 19 aa, Artificial Sequence
WIHWVRQAPGKGLEWVAWI

SEQ ID NO: 16 - protein, 19 aa, Artificial Sequence
GMHWVRQAPGKGLEWVALI

SEQ ID NO: 17 - protein, 19 aa, Artificial Sequence
GMYWVRQAPGKGQEWVAII

SEQ ID NO: 18 - protein, 19 aa, Artificial Sequence
GMHWVRQTPGKGLEWVALI

SEQ ID NO: 19 - protein, 19 aa, Artificial Sequence
DMHWVRQAPGKGLEWVAST

SEQ ID NO: 20 - protein, 19 aa, Artificial Sequence
GMYWVRQAPGKGQEWVASI

SEQ ID NO: 21 - protein, 6 aa, Artificial Sequence
SPYGGS

SEQ ID NO: 22 - protein, 6 aa, Artificial Sequence
WYDASF

SEQ ID NO: 23 - protein, 6 aa, Artificial Sequence
WYDGTK

SEQ ID NO: 24 - protein, 6 aa, Artificial Sequence
WYDGSR

SEQ ID NO: 25 - protein, 6 aa, Artificial Sequence
WYDGSN

SEQ ID NO: 26 - protein, 6 aa, Artificial Sequence
WYDASK

SEQ ID NO: 27 - protein, 6 aa, Artificial Sequence
RYTGTE

SEQ ID NO: 28 - protein, 41 aa, Artificial Sequence
TYYADSVKGRFTISADTSKNTAYLQMNSLRAEDTAVYYCAR

SEQ ID NO: 29 - protein, 41 aa, Artificial Sequence
EYYADSVKGRFSISRDNSKNTLYLQMNSLRAEDTAVYYCVR

SEQ ID NO: 30 - protein, 41 aa, Artificial Sequence
KHYADSVKGRFTISRDNSKNTLYLEMNSLRVEDTAVYYCAK

SEQ ID NO: 31 - protein, 41 aa, Artificial Sequence
KHYADSVKGRFTISRDNSKNTLYLEMNSLRAEDTAMYYCAK

SEQ ID NO: 32 - protein, 41 aa, Artificial Sequence
NYYADSVKGRFTISRDNSKNTLYLQMNSLRAEDTAVYYCAT

SEQ ID NO: 33 - protein, 41 aa, Artificial Sequence
KYYADSVKGRFTISRDNSKNTLYLQMNSLRAEDTAVYYCAK

SEQ ID NO: 34 - protein, 9 aa, Artificial Sequence
RHWPGGFDY

SEQ ID NO: 35 - protein, 10 aa, Artificial Sequence
DAQWGSRLDY

SEQ ID NO: 36 - protein, 14 aa, Artificial Sequence
NRAIFGVVPDASDI

SEQ ID NO: 37 - protein, 14 aa, Artificial Sequence
ERSSSFYYYYGMDV

SEQ ID NO: 38 - protein, 13 aa, Artificial Sequence
GGDLLTGPNAFDI

SEQ ID NO: 39 - protein, 14 aa, Artificial Sequence
NRAIFGVIPDDSDI

SEQ ID NO: 40 - protein, 14 aa, Artificial Sequence
NRALFGVIPDASDI

SEQ ID NO: 41 - protein, 14 aa, Artificial Sequence
NRALFGVIPDDSDI

SEQ ID NO: 42 - protein, 11 aa, Artificial Sequence
WGQGTLVTVSS

SEQ ID NO: 43 - protein, 11 aa, Artificial Sequence
RGQGTMVTVSS

SEQ ID NO: 44 - protein, 11 aa, Artificial Sequence
WGQGTTVTVSS

SEQ ID NO: 45 - protein, 11 aa, Artificial Sequence
WGQGTMVTVSS

SEQ ID NO: 46 - protein, 23 aa, Artificial Sequence
DIQMTQSPSSLSASVGDRVTITC

SEQ ID NO: 47 - protein, 23 aa, Artificial Sequence
KIVMTQSPATLSLSPGERATLSC

SEQ ID NO: 48 - protein, 23 aa, Artificial Sequence
DIQLTQSPSFLSTSVGDRVTITC

SEQ ID NO: 49 - protein, 23 aa, Artificial Sequence
DIQMTQSPSTLSASVGDRVTITC

SEQ ID NO: 50 - protein, 11 aa, Artificial Sequence
RASQDVSTAVA

SEQ ID NO: 51 - protein, 11 aa, Artificial Sequence
RASQSVSRYLA

SEQ ID NO: 52 - protein, 11 aa, Artificial Sequence
RASQGISSYLA

SEQ ID NO: 53 - protein, 11 aa, Artificial Sequence
RASQSISSWLA

SEQ ID NO: 54 - protein, 15 aa, Artificial Sequence
WYQQKPGKAPKLLIY

SEQ ID NO: 55 - protein, 15 aa, Artificial Sequence
WYQQKPGQAPRLLIY

SEQ ID NO: 56 - protein, 7 aa, Artificial Sequence
SASFLYS

SEQ ID NO: 57 - protein, 7 aa, Artificial Sequence
DASNRAT

SEQ ID NO: 58 - protein, 7 aa, Artificial Sequence
AASTLQS

SEQ ID NO: 59 - protein, 7 aa, Artificial Sequence
KASSLES

SEQ ID NO: 60 - protein, 32 aa, Artificial Sequence
GVPSRFSGSGSGTDFTLTISSLQPEDFATYYC

SEQ ID NO: 61 - protein, 32 aa, Artificial Sequence
GIPARFSGSGSGTDFTLTISSLEPEDFAVYYC

SEQ ID NO: 62 - protein, 32 aa, Artificial Sequence
GVPSRFSGSGSGTEFTLTISSLQPEDFATYYC

SEQ ID NO: 63 - protein, 32 aa, Artificial Sequence
GVPSRFSGSGSGTEFTLTISSLQPDDFATYYC

SEQ ID NO: 64 - protein, 9 aa, Artificial Sequence
QQYLYHPAT

SEQ ID NO: 65 - protein, 9 aa, Artificial Sequence
QQRSNWIFT

SEQ ID NO: 66 - protein, 9 aa, Artificial Sequence
QQLNSYPYT

SEQ ID NO: 67 - protein, 9 aa, Artificial Sequence
QQYDNYENT

SEQ ID NO: 68 - protein, 10 aa, Artificial Sequence
FGQGTKVEIK

SEQ ID NO: 69 - protein, 10 aa, Artificial Sequence
FGPGTKVDIK

SEQ ID NO: 70 - protein, 10 aa, Artificial Sequence
FGQGTELEIK

SEQ ID NO: 71 - protein, 10 aa, Artificial Sequence
FGQGTKLEIK

SEQ ID NO: 72 - protein, 118 aa, Artificial Sequence [sequence omitted]

SEQ ID NO: 73 - protein, 119 aa, Artificial Sequence
QVQLVESGGGVAQPGRSLSLSCAASGFTFSDYGMHWVRQAPGKGLEWVALIWYDASFEYYADSVKGRFSISRDNSKNTLYLQMNSLRAEDTAVYYCVRDAQWGSRLDYWGQGTLVTVSS

SEQ ID NO: 74 - protein, 123 aa, Artificial Sequence
QVQLVESGGGVVQPGMSLRLSCAASGFNFSNYGMYWVRQAPGKGQEWVAIIWYDGTKKHYADSVKGRFTISRDNSKNTLYLEMNSLRVEDTAVYYCAKNRAIFGVVPDASDIRGQGTMVTVSS

SEQ ID NO: 75 - protein, 123 aa, Artificial Sequence
EVQLVESGGGVVQPGRSLRLSCAASGFTFSSYGMYWVRQAPGKGQEWVAIIWYDGTKKHYADSVKGRFTISRDNSKNTLYLEMNSLRVEDTAVYYCAKNRAIFGVVPDASDIRGQGTMVTVSS

SEQ ID NO: 76 - protein, 123 aa, Artificial Sequence
EVQLLESGGGVVQPGRSLRLSCAASGFNFSSYGMYWVRQAPGKGQEWVAIIWYDGSRKHYADSVKGRFTISRDNSKNTLYLEMNSLRAEDTAMYYCAKNRAIFGVVPDASDIRGQGTMVTVSS

SEQ ID NO: 77 - protein, 123 aa, Artificial Sequence
EVQLVESGGGVVQPGRSLRLSCAASGFNFSSYGMYWVRQAPGKGQEWVAIIWYDGTKKHYADSVKGRFTISRDNSKNTLYLEMNSLRVEDTAVYYCAKNRAIFGVVPDASDIRGQGTMVTVSS

SEQ ID NO: 78 - protein, 123 aa, Artificial Sequence
QVQLVESGGGVVQPGRSLRLSCAASGFTFYSYGMHWVRQTPGKGLEWVALIWYDGSNNYYADSVKGRFTISRDNSKNTLYLQMNSLRAEDTAVYYCATERSSSFYYYYGMDVWGQGTTVTVSS

SEQ ID NO: 79 - protein, 123 aa, Artificial Sequence
QVQLVESGGGVVQPGMSLRLSCAASGFTFSNYGMYWVRQAPGKGQEWVAIIWYDGTKKHYADSVKGRFTISRDNSKNTLYLEMNSLRVEDTAVYYCAKNRAIFGVVPDASDIRGQGTMVTVSS

SEQ ID NO: 80 - protein, 123 aa, Artificial Sequence
QVQLVESGGGVVQPGMSLRLSCAASGFTFSSYGMYWVRQAPGKGQEWVAIIWYDGTKKHYADSVKGRFTISRDNSKNTLYLEMNSLRVEDTAVYYCAKNRAIFGVVPDASDIRGQGTMVTVSS

SEQ ID NO: 81 - protein, 122 aa, Artificial Sequence
QVQLVESGGGVVQPGRSLRLSCAASGFTFSSYDMHWVRQAPGKGLEWVASTWYDASKKYYADSVKGRFTISRDNSKNTLYLQMNSLRAEDTAVYYCAKGGDLLTGPNAFDIWGQGTMVTVSS

SEQ ID NO: 82 - protein, 123 aa, Artificial Sequence
QVQLVESGGGVVQPGMSLRLSCAASGFTFSSYGMYWVRQAPGKGQEWVASIRYTGTEKHYADSVKGRFTISRDNSKNTLYLEMNSLRVEDTAVYYCAKNRAIFGVVPDASDIRGQGTMVTVSS

SEQ ID NO: 83 - protein, 123 aa, Artificial Sequence
QVQLVESGGGVVQPGMSLRLSCAASGFTFSSYGMYWVRQAPGKGQEWVAIIWYDGTKKHYADSVKGRFTISRDNSKNTLYLEMNSLRVEDTAVYYCAKNRAIFGVIPDDSDIRGQGTMVTVSS

SEQ ID NO: 84 - protein, 123 aa, Artificial Sequence
QVQLVESGGGVVQPGMSLRLSCAASGFTFSSYGMYWVRQAPGKGQEWVAIIWYDGTKKHYADSVKGRFTISRDNSKNTLYLEMNSLRVEDTAVYYCAKNRALFGVIPDASDIRGQGTMVTVSS

SEQ ID NO: 85 - protein, 123 aa, Artificial Sequence
QVQLVESGGGVVQPGMSLRLSCAASGFTFSSYGMYWVRQAPGKGQEWVAIIWYDGTKKHYADSVKGRFTISRDNSKNTLYLEMNSLRVEDTAVYYCAKNRALFGVIPDDSDIRGQGTMVTVSS

SEQ ID NO: 86 - protein, 123 aa, Artificial Sequence
QVQLVESGGGVVQPGMSLRLSCAASGFTFSSYGMYWVRQAPGKGQEWVASIRYTGTEKHYADSVKGRFTISRDNSKNTLYLEMNSLRVEDTAVYYCAKNRAIFGVIPDDSDIRGQGTMVTVSS

SEQ ID NO: 87 - protein, 123 aa, Artificial Sequence
QVQLVESGGGVVQPGMSLRLSCAASGFTFSSYGMYWVRQAPGKGQEWVASIRYTGTEKHYADSVKGRFTISRDNSKNTLYLEMNSLRVEDTAVYYCAKNRALFGVIPDASDIRGQGTMVTVSS

SEQ ID NO: 88 - protein, 123 aa, Artificial Sequence
QVQLVESGGGVVQPGMSLRLSCAASGFTFSSYGMYWVRQAPGKGQEWVASIRYTGTEKHYADSVKGRFTISRDNSKNTLYLEMNSLRVEDTAVYYCAKNRALFGVIPDDSDIRGQGTMVTVSS

SEQ ID NO: 89 - protein, 123 aa, Artificial Sequence
QVQLVESGGGVVQPGMSLRLSCAASGFDFSSYGMYWVRQAPGKGQEWVASIRYTGTEKHYADSVKGRFTISRDNSKNTLYLEMNSLRVEDTAVYYCAKNRAIFGVVPDASDIRGQGTMVTVSS

SEQ ID NO: 90 - protein, 123 aa, Artificial Sequence
QVQLVESGGGVVQPGMSLRLSCAASGFDFSSYGMYWVRQAPGKGQEWVASIRYTGTEKHYADSVKGRFTISRDNSKNTLYLEMNSLRVEDTAVYYCAKNRAIFGVIPDDSDIRGQGTMVTVSS

SEQ ID NO: 91 - protein, 123 aa, Artificial Sequence
QVQLVESGGGVVQPGMSLRLSCAASGFDFSSYGMYWVRQAPGKGQEWVASIRYTGTEKHYADSVKGRFTISRDNSKNTLYLEMNSLRVEDTAVYYCAKNRALFGVIPDASDIRGQGTMVTVSS

SEQ ID NO: 92 - protein, 123 aa, Artificial Sequence
QVQLVESGGGVVQPGMSLRLSCAASGFDFSSYGMYWVRQAPGKGQEWVASIRYTGTEKHYADSVKGRFTISRDNSKNTLYLEMNSLRVEDTAVYYCAKNRALFGVIPDDSDIRGQGTMVTVSS

SEQ ID NO: 93 - protein, 107 aa, Artificial Sequence [sequence omitted]

SEQ ID NO: 94 - protein, 107 aa, Artificial Sequence
KIVMTQSPATLSLSPGERATLSCRASQSVSRYLAWYQQKPGQAPRLLIYDASNRATGIPARFSGSGSGTDFTLTISSLEPEDFAVYYCQQRSNWIFTFGPGTKVDIK

SEQ ID NO: 95 - protein, 107 aa, Artificial Sequence
DIQLTQSPSFLSTSVGDRVTITCRASQGISSYLAWYQQKPGKAPKLLIYAASTLQSGVPSRFSGSGSGTEFTLTISSLQPEDFATYYCQQLNSYPYTFGQGTELEIK

SEQ ID NO: 96 - protein, 107 aa, Artificial Sequence
DIQMTQSPSTLSASVGDRVTITCRASQSISSWLAWYQQKPGKAPKLLIYKASSLESGVPSRFSGSGSGTEFTLTISSLQPDDFATYYCQQYDNYENTFGQGTKLEIK

SEQ ID NO: 97 - protein, 448 aa, Artificial Sequence
EVQLVESGGGLVQPGGSLRLSCAASGFTFSDSWIHWVRQAPGKGLEWVAWISPYGGSTYYADSVKGRFTISADTSKNTAYLQMNSLRAEDTAVYYCARRHWPGGFDYWGQGTLVTVSSASTKGPSVFPLAPSSKSTSGGTAALGCLVKDYFPEPVTVSWNSGALTSGVHTFPAVLQSSGLYSLSSVVTVPSSSLGTQTYICNVNHKPSNTKVDKKVEPKSCDKTHTCPPCPAPELLGGPSVFLFPPKPKDTLMISRTPEVTCVVVDVSHEDPEVKFNWYVDGVEVHNAKTKPREEQYASTYRVVSVLTVLHQDWLNGKEYKCKVSNKALPAPIEKTISKAKGQPREPQVYTLPPSREEMTKNQVSLTCLVKGFYPSDIAVEWESNGQPENNYKTTPPVLDSDGSFFLYSKLTVDKSRWQQGNVFSCSVMHEALHNHYTQKSLSLSPGK

SEQ ID NO: 98 - protein, 449 aa, Artificial Sequence
QVQLVESGGGVAQPGRSLSLSCAASGFTFSDYGMHWVRQAPGKGLEWVALIWYDASFEYYADSVKGRFSISRDNSKNTLYLQMNSLRAEDTAVYYCVRDAQWGSRLDYWGQGTLVTVSSASTKGPSVFPLAPSSKSTSGGTAALGCLVKDYFPEPVTVSWNSGALTSGVHTFPAVLQSSGLYSLSSVVTVPSSSLGTQTYICNVNHKPSNTKVDKKVEPKSCDKTHTCPPCPAPEAAGGPSVFLFPPKPKDTLMISRTPEVTCVVVDVSHEDPEVKFNWYVDGVEVHNAKTKPREEQYNSTYRVVSVLTVLHQDWLNGKEYKCKVSNKALPAPIEKTISKAKGQPREPQVYTLPPSREEMTKNQVSLTCLVKGFYPSDIAVEWESNGQPENNYKTTPPVLDSDGSFFLYSKLTVDKSRWQQGNVFSCSVMHEALHNHYTQKSLSLSPGK

SEQ ID NO: 99 - protein, 355 aa, Artificial Sequence
QVQLVESGGGVVQPGMSLRLSCAASGFNFSNYGMYWVRQAPGKGQEWVAIIWYDGTKKHYADSVKGRFTISRDNSKNTLYLEMNSLRVEDTAVYYCAKNRAIFGVVPDASDIRGQGTMVTVSSEPKSCDKTHTCPPCPAPELLGGPSVFLFPPKPKDTLMISRTPEVTCVVVDVSHEDPEVKFNWYVDGVEVHNAKTKPREEQYNSTYRVVSVLTVLHQDWLNGKEYKCKVSNKALPAPIEKTISKAKGQPREPQVYTLPPSREEMTKNQVSLTCLVKGFYPSDIAVEWESNGQPENNYKTTPPVLDSDGSFFLYSKLTVDKSRWQQGNVFSCSVMHEALHNHYTQKSLSLSPGK

SEQ ID NO: 100 - protein, 355 aa, Artificial Sequence
EVQLVESGGGVVQPGRSLRLSCAASGFTFSSYGMYWVRQAPGKGQEWVAIIWYDGTKKHYADSVKGRFTISRDNSKNTLYLEMNSLRVEDTAVYYCAKNRAIFGVVPDASDIRGQGTMVTVSSEPKSCDKTHTCPPCPAPELLGGPSVFLFPPKPKDTLMISRTPEVTCVVVDVSHEDPEVKFNWYVDGVEVHNAKTKPREEQYNSTYRVVSVLTVLHQDWLNGKEYKCKVSNKALPAPIEKTISKAKGQPREPQVYTLPPSREEMTKNQVSLTCLVKGFYPSDIAVEWESNGQPENNYKTTPPVLDSDGSFFLYSKLTVDKSRWQQGNVFSCSVMHEALHNHYTQKSLSLSPGK

SEQ ID NO: 101 - protein, 355 aa, Artificial Sequence
EVQLLESGGGVVQPGRSLRLSCAASGFNFSSYGMYWVRQAPGKGQEWVAIIWYDGSRKHYADSVKGRFTISRDNSKNTLYLEMNSLRAEDTAMYYCAKNRAIFGVVPDASDIRGQGTMVTVSSEPKSCDKTHTCPPCPAPELLGGPSVFLFPPKPKDTLMISRTPEVTCVVVDVSHEDPEVKFNWYVDGVEVHNAKTKPREEQYNSTYRVVSVLTVLHQDWLNGKEYKCKVSNKALPAPIEKTISKAKGQPREPQVYTLPPSREEMTKNQVSLTCLVKGFYPSDIAVEWESNGQPENNYKTTPPVLDSDGSFFLYSKLTVDKSRWQQGNVFSCSVMHEALHNHYTQKSLSLSPGK

SEQ ID NO: 102 - protein, 355 aa, Artificial Sequence
EVQLVESGGGVVQPGRSLRLSCAASGFNFSSYGMYWVRQAPGKGQEWVAIIWYDGTKKHYADSVKGRFTISRDNSKNTLYLEMNSLRVEDTAVYYCAKNRAIFGVVPDASDIRGQGTMVTVSSEPKSCDKTHTCPPCPAPELLGGPSVFLFPPKPKDTLMISRTPEVTCVVVDVSHEDPEVKFNWYVDGVEVHNAKTKPREEQYNSTYRVVSVLTVLHQDWLNGKEYKCKVSNKALPAPIEKTISKAKGQPREPQVYTLPPSREEMTKNQVSLTCLVKGFYPSDIAVEWESNGQPENNYKTTPPVLDSDGSFFLYSKLTVDKSRWQQGNVFSCSVMHEALHNHYTQKSLSLSPGK

SEQ ID NO: 103 - protein, 453 aa, Artificial Sequence
QVQLVESGGGVVQPGRSLRLSCAASGFTFYSYGMHWVRQTPGKGLEWVALIWYDGSNNYYADSVKGRFTISRDNSKNTLYLQMNSLRAEDTAVYYCATERSSSFYYYYGMDVWGQGTTVTVSSASTKGPSVFPLAPSSKSTSGGTAALGCLVKDYFPEPVTVSWNSGALTSGVHTFPAVLQSSGLYSLSSVVTVPSSSLGTQTYICNVNHKPSNTKVDKKVEPKSCDKTHTCPPCPAPEAAGGPSVFLFPPKPKDTLMISRTPEVTCVVVDVSHEDPEVKFNWYVDGVEVHNAKTKPREEQYNSTYRVVSVLTVLHQDWLNGKEYKCKVSNKALPAPIEKTISKAKGQPREPQVYTLPPSREEMTKNQVSLTCLVKGFYPSDIAVEWESNGQPENNYKTTPPVLDSDGSFFLYSKLTVDKSRWQQGNVFSCSVMHEALHNHYTQKSLSLSPGK

SEQ ID NO: 104 - protein, 355 aa, Artificial Sequence
QVQLVESGGGVVQPGMSLRLSCAASGFTFSNYGMYWVRQAPGKGQEWVAIIWYDGTKKHYADSVKGRFTISRDNSKNTLYLEMNSLRVEDTAVYYCAKNRAIFGVVPDASDIRGQGTMVTVSSEPKSCDKTHTCPPCPAPELLGGPSVFLFPPKPKDTLMISRTPEVTCVVVDVSHEDPEVKFNWYVDGVEVHNAKTKPREEQYNSTYRVVSVLTVLHQDWLNGKEYKCKVSNKALPAPIEKTISKAKGQPREPQVYTLPPSREEMTKNQVSLTCLVKGFYPSDIAVEWESNGQPENNYKTTPPVLDSDGSFFLYSKLTVDKSRWQQGNVFSCSVMHEALHNHYTQKSLSLSPGK

SEQ ID NO: 105 - protein, 355 aa, Artificial Sequence
QVQLVESGGGVVQPGMSLRLSCAASGFTFSSYGMYWVRQAPGKGQEWVAIIWYDGTKKHYADSVKGRFTISRDNSKNTLYLEMNSLRVEDTAVYYCAKNRAIFGVVPDASDIRGQGTMVTVSSEPKSCDKTHTCPPCPAPELLGGPSVFLFPPKPKDTLMISRTPEVTCVVVDVSHEDPEVKFNWYVDGVEVHNAKTKPREEQYNSTYRVVSVLTVLHQDWLNGKEYKCKVSNKALPAPIEKTISKAKGQPREPQVYTLPPSREEMTKNQVSLTCLVKGFYPSDIAVEWESNGQPENNYKTTPPVLDSDGSFFLYSKLTVDKSRWQQGNVFSCSVMHEALHNHYTQKSLSLSPGK

SEQ ID NO: 106 - protein, 452 aa, Artificial Sequence
QVQLVESGGGVVQPGRSLRLSCAASGFTFSSYDMHWVRQAPGKGLEWVASTWYDASKKYYADSVKGRFTISRDNSKNTLYLQMNSLRAEDTAVYYCAKGGDLLTGPNAFDIWGQGTMVTVSSASTKGPSVFPLAPSSKSTSGGTAALGCLVKDYFPEPVTVSWNSGALTSGVHTFPAVLQSSGLYSLSSVVTVPSSSLGTQTYICNVNHKPSNTKVDKKVEPKSCDKTHTCPPCPAPEAAGGPSVFLFPPKPKDTLMISRTPEVTCVVVDVSHEDPEVKFNWYVDGVEVHNAKTKPREEQYNSTYRVVSVLTVLHQDWLNGKEYKCKVSNKALPAPIEKTISKAKGQPREPQVYTLPPSREEMTKNQVSLTCLVKGFYPSDIAVEWESNGQPENNYKTTPPVLDSDGSFFLYSKLTVDKSRWQQGNVFSCSVMHEALHNHYTQKSLSLSPGK

SEQ ID NO: 107 - protein, 355 aa, Artificial Sequence
QVQLVESGGGVVQPGMSLRLSCAASGFTFSSYGMYWVRQAPGKGQEWVASIRYTGTEKHYADSVKGRFTISRDNSKNTLYLEMNSLRVEDTAVYYCAKNRAIFGVVPDASDIRGQGTMVTVSSEPKSCDKTHTCPPCPAPELLGGPSVFLFPPKPKDTLMISRTPEVTCVVVDVSHEDPEVKFNWYVDGVEVHNAKTKPREEQYNSTYRVVSVLTVLHQDWLNGKEYKCKVSNKALPAPIEKTISKAKGQPREPQVYTLPPSREEMTKNQVSLTCLVKGFYPSDIAVEWESNGQPENNYKTTPPVLDSDGSFFLYSKLTVDKSRWQQGNVFSCSVMHEALHNHYTQKSLSLSPGK

SEQ ID NO: 108 - protein, 355 aa, Artificial Sequence
QVQLVESGGGVVQPGMSLRLSCAASGFTFSSYGMYWVRQAPGKGQEWVAIIWYDGTKKHYADSVKGRFTISRDNSKNTLYLEMNSLRVEDTAVYYCAKNRAIFGVIPDDSDIRGQGTMVTVSSEPKSCDKTHTCPPCPAPELLGGPSVFLFPPKPKDTLMISRTPEVTCVVVDVSHEDPEVKFNWYVDGVEVHNAKTKPREEQYNSTYRVVSVLTVLHQDWLNGKEYKCKVSNKALPAPIEKTISKAKGQPREPQVYTLPPSREEMTKNQVSLTCLVKGFYPSDIAVEWESNGQPENNYKTTPPVLDSDGSFFLYSKLTVDKSRWQQGNVFSCSVMHEALHNHYTQKSLSLSPGK

SEQ ID NO: 109 - protein, 355 aa, Artificial Sequence
QVQLVESGGGVVQPGMSLRLSCAASGFTFSSYGMYWVRQAPGKGQEWVAIIWYDGTKKHYADSVKGRFTISRDNSKNTLYLEMNSLRVEDTAVYYCAKNRALFGVIPDASDIRGQGTMVTVSSEPKSCDKTHTCPPCPAPELLGGPSVFLFPPKPKDTLMISRTPEVTCVVVDVSHEDPEVKFNWYVDGVEVHNAKTKPREEQYNSTYRVVSVLTVLHQDWLNGKEYKCKVSNKALPAPIEKTISKAKGQPREPQVYTLPPSREEMTKNQVSLTCLVKGFYPSDIAVEWESNGQPENNYKTTPPVLDSDGSFFLYSKLTVDKSRWQQGNVFSCSVMHEALHNHYTQKSLSLSPGK

SEQ ID NO: 110 - protein, 355 aa, Artificial Sequence
QVQLVESGGGVVQPGMSLRLSCAASGFTFSSYGMYWVRQAPGKGQEWVAIIWYDGTKKHYADSVKGRFTISRDNSKNTLYLEMNSLRVEDTAVYYCAKNRALFGVIPDDSDIRGQGTMVTVSSEPKSCDKTHTCPPCPAPELLGGPSVFLFPPKPKDTLMISRTPEVTCVVVDVSHEDPEVKFNWYVDGVEVHNAKTKPREEQYNSTYRVVSVLTVLHQDWLNGKEYKCKVSNKALPAPIEKTISKAKGQPREPQVYTLPPSREEMTKNQVSLTCLVKGFYPSDIAVEWESNGQPENNYKTTPPVLDSDGSFFLYSKLTVDKSRWQQGNVFSCSVMHEALHNHYTQKSLSLSPGK

SEQ ID NO: 111 - protein, 355 aa, Artificial Sequence
QVQLVESGGGVVQPGMSLRLSCAASGFTFSSYGMYWVRQAPGKGQEWVASIRYTGTEKHYADSVKGRFTISRDNSKNTLYLEMNSLRVEDTAVYYCAKNRAIFGVIPDDSDIRGQGTMVTVSSEPKSCDKTHTCPPCPAPELLGGPSVFLFPPKPKDTLMISRTPEVTCVVVDVSHEDPEVKFNWYVDGVEVHNAKTKPREEQYNSTYRVVSVLTVLHQDWLNGKEYKCKVSNKALPAPIEKTISKAKGQPREPQVYTLPPSREEMTKNQVSLTCLVKGFYPSDIAVEWESNGQPENNYKTTPPVLDSDGSFFLYSKLTVDKSRWQQGNVFSCSVMHEALHNHYTQKSLSLSPGK

SEQ ID NO: 112 - protein, 355 aa, Artificial Sequence
QVQLVESGGGVVQPGMSLRLSCAASGFTFSSYGMYWVRQAPGKGQEWVASIRYTGTEKHYADSVKGRFTISRDNSKNTLYLEMNSLRVEDTAVYYCAKNRALFGVIPDASDIRGQGTMVTVSSEPKSCDKTHTCPPCPAPELLGGPSVFLFPPKPKDTLMISRTPEVTCVVVDVSHEDPEVKFNWYVDGVEVHNAKTKPREEQYNSTYRVVSVLTVLHQDWLNGKEYKCKVSNKALPAPIEKTISKAKGQPREPQVYTLPPSREEMTKNQVSLTCLVKGFYPSDIAVEWESNGQPENNYKTTPPVLDSDGSFFLYSKLTVDKSRWQQGNVFSCSVMHEALHNHYTQKSLSLSPGK

SEQ ID NO: 113 - protein, 355 aa, Artificial Sequence
QVQLVESGGGVVQPGMSLRLSCAASGFTFSSYGMYWVRQAPGKGQEWVASIRYTGTEKHYADSVKGRFTISRDNSKNTLYLEMNSLRVEDTAVYYCAKNRALFGVIPDDSDIRGQGTMVTVSSEPKSCDKTHTCPPCPAPELLGGPSVFLFPPKPKDTLMISRTPEVTCVVVDVSHEDPEVKFNWYVDGVEVHNAKTKPREEQYNSTYRVVSVLTVLHQDWLNGKEYKCKVSNKALPAPIEKTISKAKGQPREPQVYTLPPSREEMTKNQVSLTCLVKGFYPSDIAVEWESNGQPENNYKTTPPVLDSDGSFFLYSKLTVDKSRWQQGNVFSCSVMHEALHNHYTQKSLSLSPGK

SEQ ID NO: 114 - protein, 355 aa, Artificial Sequence
QVQLVESGGGVVQPGMSLRLSCAASGFDFSSYGMYWVRQAPGKGQEWVASIRYTGTEKHYADSVKGRFTISRDNSKNTLYLEMNSLRVEDTAVYYCAKNRAIFGVVPDASDIRGQGTMVTVSSEPKSCDKTHTCPPCPAPELLGGPSVFLFPPKPKDTLMISRTPEVTCVVVDVSHEDPEVKFNWYVDGVEVHNAKTKPREEQYNSTYRVVSVLTVLHQDWLNGKEYKCKVSNKALPAPIEKTISKAKGQPREPQVYTLPPSREEMTKNQVSLTCLVKGFYPSDIAVEWESNGQPENNYKTTPPVLDSDGSFFLYSKLTVDKSRWQQGNVFSCSVMHEALHNHYTQKSLSLSPGK

SEQ ID NO: 115 - protein, 355 aa, Artificial Sequence
QVQLVESGGGVVQPGMSLRLSCAASGFDFSSYGMYWVRQAPGKGQEWVASIRYTGTEKHYADSVKGRFTISRDNSKNTLYLEMNSLRVEDTAVYYCAKNRAIFGVIPDDSDIRGQGTMVTVSSEPKSCDKTHTCPPCPAPELLGGPSVFLFPPKPKDTLMISRTPEVTCVVVDVSHEDPEVKFNWYVDGVEVHNAKTKPREEQYNSTYRVVSVLTVLHQDWLNGKEYKCKVSNKALPAPIEKTISKAKGQPREPQVYTLPPSREEMTKNQVSLTCLVKGFYPSDIAVEWESNGQPENNYKTTPPVLDSDGSFFLYSKLTVDKSRWQQGNVFSCSVMHEALHNHYTQKSLSLSPGK

SEQ ID NO: 116 - protein, 355 aa, Artificial Sequence
QVQLVESGGGVVQPGMSLRLSCAASGFDFSSYGMYWVRQAPGKGQEWVASIRYTGTEKHYADSVKGRFTISRDNSKNTLYLEMNSLRVEDTAVYYCAKNRALFGVIPDASDIRGQGTMVTVSSEPKSCDKTHTCPPCPAPELLGGPSVFLFPPKPKDTLMISRTPEVTCVVVDVSHEDPEVKFNWYVDGVEVHNAKTKPREEQYNSTYRVVSVLTVLHQDWLNGKEYKCKVSNKALPAPIEKTISKAKGQPREPQVYTLPPSREEMTKNQVSLTCLVKGFYPSDIAVEWESNGQPENNYKTTPPVLDSDGSFFLYSKLTVDKSRWQQGNVFSCSVMHEALHNHYTQKSLSLSPGK

SEQ ID NO: 117 - protein, 355 aa, Artificial Sequence
QVQLVESGGGVVQPGMSLRLSCAASGFDFSSYGMYWVRQAPGKGQEWVASIRYTGTEKHYADSVKGRFTISRDNSKNTLYLEMNSLRVEDTAVYYCAKNRALFGVIPDDSDIRGQGTMVTVSSEPKSCDKTHTCPPCPAPELLGGPSVFLFPPKPKDTLMISRTPEVTCVVVDVSHEDPEVKFNWYVDGVEVHNAKTKPREEQYNSTYRVVSVLTVLHQDWLNGKEYKCKVSNKALPAPIEKTISKAKGQPREPQVYTLPPSREEMTKNQVSLTCLVKGFYPSDIAVEWESNGQPENNYKTTPPVLDSDGSFFLYSKLTVDKSRWQQGNVFSCSVMHEALHNHYTQKSLSLSPGK

SEQ ID NO: 118 - protein, 214 aa, Artificial Sequence
DIQMTQSPSSLSASVGDRVTITCRASQDVSTAVAWYQQKPGKAPKLLIYSASFLYSGVPSRFSGSGSGTDFTLTISSLQPEDFATYYCQQYLYHPATFGQGTKVEIKRTVAAPSVFIFPPSDEQLKSGTASVVCLLNNFYPREAKVQWKVDNALQSGNSQESVTEQDSKDSTYSLSSTLTLSKADYEKHKVYACEVTHQGLSSPVTKSFNRGEC

SEQ ID NO: 119 - protein, 214 aa, Artificial Sequence
KIVMTQSPATLSLSPGERATLSCRASQSVSRYLAWYQQKPGQAPRLLIYDASNRATGIPARFSGSGSGTDFTLTISSLEPEDFAVYYCQQRSNWIFTFGPGTKVDIKRTVAAPSVFIFPPSDEQLKSGTASVVCLLNNFYPREAKVQWKVDNALQSGNSQESVTEQDSKDSTYSLSSTLTLSKADYEKHKVYACEVTHQGLSSPVTKSFNRGEC

SEQ ID NO: 120 - protein, 214 aa, Artificial Sequence
DIQLTQSPSFLSTSVGDRVTITCRASQGISSYLAWYQQKPGKAPKLLIYAASTLQSGVPSRFSGSGSGTEFTLTISSLQPEDFATYYCQQLNSYPYTFGQGTELEIKRTVAAPSVFIFPPSDEQLKSGTASVVCLLNNFYPREAKVQWKVDNALQSGNSQESVTEQDSKDSTYSLSSTLTLSKADYEKHKVYACEVTHQGLSSPVTKSFNRGEC

SEQ ID NO: 121 - protein, 214 aa, Artificial Sequence
DIQMTQSPSTLSASVGDRVTITCRASQSISSWLAWYQQKPGKAPKLLIYKASSLESGVPSRFSGSGSGTEFTLTISSLQPDDFATYYCQQYDNYENTFGQGTKLEIKRTVAAPSVFIFPPSDEQLKSGTASVVCLLNNFYPREAKVQWKVDNALQSGNSQESVTEQDSKDSTYSLSSTLTLSKADYEKHKVYACEVTHQGLSSPVTKSFNRGEC

SEQ ID NO: 122 - protein, 587 aa, Artificial Sequence
QVQLVESGGGVVQPGMSLRLSCAASGFTFSSYGMYWVRQAPGKGQEWVAIIWYDGTKKHYADSVKGRFTISRDNSKNTLYLEMNSLRVEDTAVYYCAKNRAIFGVVPDASDIRGQGTMVTVSSGGGGSGGGGSGGGGSQVQLVESGGGVAQPGRSLSLSCAASGFTFSDYGMHWVRQAPGKGLEWVALIWYDASFEYYADSVKGRFSISRDNSKNTLYLQMNSLRAEDTAVYYCVRDAQWGSRLDYWGQGTLVTVSSASTKGPSVFPLAPSSKSTSGGTAALGCLVKDYFPEPVTVSWNSGALTSGVHTFPAVLQSSGLYSLSSVVTVPSSSLGTQTYICNVNHKPSNTKVDKKVEPKSCDKTHTCPPCPAPEAAGGPSVFLFPPKPKDTLMISRTPEVTCVVVDVSHEDPEVKFNWYVDGVEVHNAKTKPREEQYNSTYRVVSVLTVLHQDWLNGKEYKCKVSNKALPAPIEKTISKAKGQPREPQVYTLPPSREEMTKNQVSLTCLVKGFYPSDIAVEWESNGQPENNYKTTPPVLDSDGSFFLYSKLTVDKSRWQQGNVFSCSVMHEALHNHYTQKSLSLSPGK

SEQ ID NO: 123 - protein, 591 aa, Artificial Sequence
QVQLVESGGGVVQPGMSLRLSCAASGFTFSSYGMYWVRQAPGKGQEWVAIIWYDGTKKHYADSVKGRFTISRDNSKNTLYLEMNSLRVEDTAVYYCAKNRAIFGVVPDASDIRGQGTMVTVSSGGGGSGGGGSGGGGSQVQLVESGGGVVQPGRSLRLSCAASGFTFYSYGMHWVRQTPGKGLEWVALIWYDGSNNYYADSVKGRFTISRDNSKNTLYLQMNSLRAEDTAVYYCATERSSSFYYYYGMDVWGQGTTVTVSSASTKGPSVFPLAPSSKSTSGGTAALGCLVKDYFPEPVTVSWNSGALTSGVHTFPAVLQSSGLYSLSSVVTVPSSSLGTQTYICNVNHKPSNTKVDKKVEPKSCDKTHTCPPCPAPEAAGGPSVFLFPPKPKDTLMISRTPEVTCVVVDVSHEDPEVKFNWYVDGVEVHNAKTKPREEQYNSTYRVVSVLTVLHQDWLNGKEYKCKVSNKALPAPIEKTISKAKGQPREPQVYTLPPSREEMTKNQVSLTCLVKGFYPSDIAVEWESNGQPENNYKTTPPVLDSDGSFFLYSKLTVDKSRWQQGNVFSCSVMHEALHNHYTQKSLSLSPGK

SEQ ID NO: 124 - protein, 590 aa, Artificial Sequence
QVQLVESGGGVVQPGMSLRLSCAASGFTFSSYGMYWVRQAPGKGQEWVAIIWYDGTKKHYADSVKGRFTISRDNSKNTLYLEMNSLRVEDTAVYYCAKNRAIFGVVPDASDIRGQGTMVTVSSGGGGSGGGGSGGGGSQVQLVESGGGVVQPGRSLRLSCAASGFTFSSYDMHWVRQAPGKGLEWVASTWYDASKKYYADSVKGRFTISRDNSKNTLYLQMNSLRAEDTAVYYCAKGGDLLTGPNAFDIWGQGTMVTVSSASTKGPSVFPLAPSSKSTSGGTAALGCLVKDYFPEPVTVSWNSGALTSGVHTFPAVLQSSGLYSLSSVVTVPSSSLGTQTYICNVNHKPSNTKVDKKVEPKSCDKTHTCPPCPAPEAAGGPSVFLFPPKPKDTLMISRTPEVTCVVVDVSHEDPEVKFNWYVDGVEVHNAKTKPREEQYNSTYRVVSVLTVLHQDWLNGKEYKCKVSNKALPAPIEKTISKAKGQPREPQVYTLPPSREEMTKNQVSLTCLVKGFYPSDIAVEWESNGQPENNYKTTPPVLDSDGSFFLYSKLTVDKSRWQQGNVFSCSVMHEALHNHYTQKSLSLSPGK

SEQ ID NO: 125 - protein, 587 aa, Artificial Sequence
QVQLVESGGGVVQPGMSLRLSCAASGFTFSSYGMYWVRQAPGKGQEWVASIRYTGTEKHYADSVKGRFTISRDNSKNTLYLEMNSLRVEDTAVYYCAKNRAIFGVVPDASDIRGQGTMVTVSSGGGGSGGGGSGGGGSQVQLVESGGGVAQPGRSLSLSCAASGFTFSDYGMHWVRQAPGKGLEWVALIWYDASFEYYADSVKGRFSISRDNSKNTLYLQMNSLRAEDTAVYYCVRDAQWGSRLDYWGQGTLVTVSSASTKGPSVFPLAPSSKSTSGGTAALGCLVKDYFPEPVTVSWNSGALTSGVHTFPAVLQSSGLYSLSSVVTVPSSSLGTQTYICNVNHKPSNTKVDKKVEPKSCDKTHTCPPCPAPEAAGGPSVFLFPPKPKDTLMISRTPEVTCVVVDVSHEDPEVKFNWYVDGVEVHNAKTKPREEQYNSTYRVVSVLTVLHQDWLNGKEYKCKVSNKALPAPIEKTISKAKGQPREPQVYTLPPSREEMTKNQVSLTCLVKGFYPSDIAVEWESNGQPENNYKTTPPVLDSDGSFFLYSKLTVDKSRWQQGNVFSCSVMHEALHNHYTQKSLSLSPGK

SEQ ID NO: 126 - protein, 587 aa, Artificial Sequence
QVQLVESGGGVVQPGMSLRLSCAASGFTFSSYGMYWVRQAPGKGQEWVASIRYTGTEKHYADSVKGRFTISRDNSKNTLYLEMNSLRVEDTAVYYCAKNRAIFGVIPDDSDIRGQGTMVTVSSGGGGSGGGGSGGGGSQVQLVESGGGVAQPGRSLSLSCAASGFTFSDYGMHWVRQAPGKGLEWVALIWYDASFEYYADSVKGRFSISRDNSKNTLYLQMNSLRAEDTAVYYCVRDAQWGSRLDYWGQGTLVTVSSASTKGPSVFPLAPSSKSTSGGTAALGCLVKDYFPEPVTVSWNSGALTSGVHTFPAVLQSSGLYSLSSVVTVPSSSLGTQTYICNVNHKPSNTKVDKKVEPKSCDKTHTCPPCPAPEAAGGPSVFLFPPKPKDTLMISRTPEVTCVVVDVSHEDPEVKFNWYVDGVEVHNAKTKPREEQYNSTYRVVSVLTVLHQDWLNGKEYKCKVSNKALPAPIEKTISKAKGQPREPQVYTLPPSREEMTKNQVSLTCLVKGFYPSDIAVEWESNGQPENNYKTTPPVLDSDGSFFLYSKLTVDKSRWQQGNVFSCSVMHEALHNHYTQKSLSLSPGK

SEQ ID NO: 127 - protein, 587 aa, Artificial Sequence
QVQLVESGGGVVQPGMSLRLSCAASGFTFSSYGMYWVRQAPGKGQEWVASIRYTGTEKHYADSVKGRFTISRDNSKNTLYLEMNSLRVEDTAVYYCAKNRALFGVIPDASDIRGQGTMVTVSSGGGGSGGGGSGGGGSQVQLVESGGGVAQPGRSLSLSCAASGFTFSDYGMHWVRQAPGKGLEWVALIWYDASFEYYADSVKGRFSISRDNSKNTLYLQMNSLRAEDTAVYYCVRDAQWGSRLDYWGQGTLVTVSSASTKGPSVFPLAPSSKSTSGGTAALGCLVKDYFPEPVTVSWNSGALTSGVHTFPAVLQSSGLYSLSSVVTVPSSSLGTQTYICNVNHKPSNTKVDKKVEPKSCDKTHTCPPCPAPEAAGGPSVFLFPPKPKDTLMISRTPEVTCVVVDVSHEDPEVKFNWYVDGVEVHNAKTKPREEQYNSTYRVVSVLTVLHQDWLNGKEYKCKVSNKALPAPIEKTISKAKGQPREPQVYTLPPSREEMTKNQVSLTCLVKGFYPSDIAVEWESNGQPENNYKTTPPVLDSDGSFFLYSKLTVDKSRWQQGNVFSCSVMHEALHNHYTQKSLSLSPGK

SEQ ID NO: 128 - protein, 587 aa, Artificial Sequence
QVQLVESGGGVVQPGMSLRLSCAASGFTFSSYGMYWVRQAPGKGQEWVASIRYTGTEKHYADSVKGRFTISRDNSKNTLYLEMNSLRVEDTAVYYCAKNRALFGVIPDDSDIRGQGTMVTVSSGGGGSGGGGSGGGGSQVQLVESGGGVAQPGRSLSLSCAASGFTFSDYGMHWVRQAPGKGLEWVALIWYDASFEYYADSVKGRFSISRDNSKNTLYLQMNSLRAEDTAVYYCVRDAQWGSRLDYWGQGTLVTVSSASTKGPSVFPLAPSSKSTSGGTAALGCLVKDYFPEPVTVSWNSGALTSGVHTFPAVLQSSGLYSLSSVVTVPSSSLGTQTYICNVNHKPSNTKVDKKVEPKSCDKTHTCPPCPAPEAAGGPSVFLFPPKPKDTLMISRTPEVTCVVVDVSHEDPEVKFNWYVDGVEVHNAKTKPREEQYNSTYRVVSVLTVLHQDWLNGKEYKCKVSNKALPAPIEKTISKAKGQPREPQVYTLPPSREEMTKNQVSLTCLVKGFYPSDIAVEWESNGQPENNYKTTPPVLDSDGSFFLYSKLTVDKSRWQQGNVFSCSVMHEALHNHYTQKSLSLSPGK

SEQ ID NO: 129 - protein, 577 aa, Artificial Sequence
QVQLVESGGGVAQPGRSLSLSCAASGFTFSDYGMHWVRQAPGKGLEWVALIWYDASFEYYADSVKGRFSISRDNSKNTLYLQMNSLRAEDTAVYYCVRDAQWGSRLDYWGQGTLVTVSSASTKGPSVFPLAPSSKSTSGGTAALGCLVKDYFPEPVTVSWNSGALTSGVHTFPAVLQSSGLYSLSSVVTVPSSSLGTQTYICNVNHKPSNTKVDKKVEPKSCDKTHTCPPCPAPEAAGAPSVFLFPPKPKDTLMISRTPEVTCVVVDVSHEDPEVKFNWYVDGVEVHNAKTKPREEQYNSTYRVVSVLTVLHQDWLNGKEYKCKVSNKALPAPIEKTISKAKGQPREPQVYTLPPSREEMTKNQVSLTCLVKGFYPSDIAVEWESNGQPENNYKTTPPVLDSDGSFFLYSKLTVDKSRWQQGNVFSCSVMHEALHNHYTQKSLSLSPGGGSGGSQVQLVESGGGVVQPGMSLRLSCAASGFDFSSYGMYWVRQAPGKGQEWVASIRYTGTEKHYADSVKGRFTISRDNSKNTLYLEMNSLRVEDTAVYYCAKNRAIFGVIPDDSDIRGQGTMVTVSS

SEQ ID NO: 130 - protein, 577 aa, Artificial Sequence
QVQLVESGGGVAQPGRSLSLSCAASGFTFSDYGMHWVRQAPGKGLEWVALIWYDASFEYYADSVKGRFSISRDNSKNTLYLQMNSLRAEDTAVYYCVRDAQWGSRLDYWGQGTLVTVSSASTKGPSVFPLAPSSKSTSGGTAALGCLVKDYFPEPVTVSWNSGALTSGVHTFPAVLQSSGLYSLSSVVTVPSSSLGTQTYICNVNHKPSNTKVDKKVEPKSCDKTHTCPPCPAPEAAGAPSVFLFPPKPKDTLMISRTPEVTCVVVDVSHEDPEVKFNWYVDGVEVHNAKTKPREEQYNSTYRVVSVLTVLHQDWLNGKEYKCKVSNKALPAPIEKTISKAKGQPREPQVYTLPPSREEMTKNQVSLTCLVKGFYPSDIAVEWESNGQPENNYKTTPPVLDSDGSFFLYSKLTVDKSRWQQGNVFSCSVMHEALHNHYTQKSLSLSPGGGSGGSQVQLVESGGGVVQPGMSLRLSCAASGFDFSSYGMYWVRQAPGKGQEWVASIRYTGTEKHYADSVKGRFTISRDNSKNTLYLEMNSLRVEDTAVYYCAKNRALFGVIPDDSDIRGQGTMVTVSS

SEQ ID NO: 131 - protein, 222 aa, Artificial Sequence
QVQLVESGGGVAQPGRSLSLSCAASGFTFSDYGMHWVRQAPGKGLEWVALIWYDASFEYYADSVKGRFSISRDNSKNTLYLQMNSLRAEDTAVYYCVRDAQWGSRLDYWGQGTLVTVSSASTKGPSVFPLAPSSKSTSGGTAALGCLVKDYFPEPVTVSWNSGALTSGVHTFPAVLQSSGLYSLSSVVTVPSSSLGTQTYICNVNHKPSNTKVDKKVEPKSC

SEQ ID NO: 132 - protein, 569 aa, Artificial Sequence
KIVMTQSPATLSLSPGERATLSCRASQSVSRYLAWYQQKPGQAPRLLIYDASNRATGIPARFSGSGSGTDFTLTISSLEPEDFAVYYCQQRSNWIFTFGPGTKVDIKRTVAAPSVFIFPPSDEQLKSGTASVVCLLNNFYPREAKVQWKVDNALQSGNSQESVTEQDSKDSTYSLSSTLTLSKADYEKHKVYACEVTHQGLSSPVTKSFNRGECQVQLVESGGGVVQPGMSLRLSCAASGFDFSSYGMYWVRQAPGKGQEWVASIRYTGTEKHYADSVKGRFTISRDNSKNTLYLEMNSLRVEDTAVYYCAKNRAIFGVIPDDSDIRGQGTMVTVSSEPKSSDKTHTCPPCPAPEAAGAPSVFLFPPKPKDTLMISRTPEVTCVVVDVSHEDPEVKFNWYVDGVEVHNAKTKPREEQYNSTYRVVSVLTVLHQDWLNGKEYKCKVSNKALPAPIEKTISKAKGQPREPQVYTLPPSREEMTKNQVSLTCLVKGFYPSDIAVEWESNGQPENNYKTTPPVLDSDGSFFLYSKLTVDKSRWQQGNVFSCSVMHEALHNHYTQKSLSLSPGK

SEQ ID NO: 133 - protein, 569 aa, Artificial Sequence
KIVMTQSPATLSLSPGERATLSCRASQSVSRYLAWYQQKPGQAPRLLIYDASNRATGIPARFSGSGSGTDFTLTISSLEPEDFAVYYCQQRSNWIFTFGPGTKVDIKRTVAAPSVFIFPPSDEQLKSGTASVVCLLNNFYPREAKVQWKVDNALQSGNSQESVTEQDSKDSTYSLSSTLTLSKADYEKHKVYACEVTHQGLSSPVTKSFNRGECQVQLVESGGGVVQPGMSLRLSCAASGFDFSSYGMYWVRQAPGKGQEWVASIRYTGTEKHYADSVKGRFTISRDNSKNTLYLEMNSLRVEDTAVYYCAKNRALFGVIPDDSDIRGQGTMVTVSSEPKSSDKTHTCPPCPAPEAAGAPSVFLFPPKPKDTLMISRTPEVTCVVVDVSHEDPEVKFNWYVDGVEVHNAKTKPREEQYNSTYRVVSVLTVLHQDWLNGKEYKCKVSNKALPAPIEKTISKAKGQPREPQVYTLPPSREEMTKNQVSLTCLVKGFYPSDIAVEWESNGQPENNYKTTPPVLDSDGSFFLYSKLTVDKSRWQQGNVFSCSVMHEALHNHYTQKSLSLSPGK

SEQ ID NO: 134 - DNA, 24 bp, Artificial Sequence
ggtgtccagtgtsaggtgcagctg

SEQ ID NO: 135 - DNA, 29 bp, Artificial Sequence
aatccctgggcactgaagagacggtgacc

SEQ ID NO: 136 - protein, 4 aa, Artificial Sequence
GSGS

SEQ ID NO: 137 - protein, 5 aa, Artificial Sequence
GGGGS

SEQ ID NO: 138 - protein, 6 aa, Artificial Sequence
GGSGGS

SEQ ID NO: 139 - protein, 7 aa, Artificial Sequence
GGGGSGS

SEQ ID NO: 140 - protein, 15 aa, Artificial Sequence
GGGGSGGGGSGGGGS

SEQ ID NO: 141 - protein, 20 aa, Artificial Sequence
GGGGSGGGGSGGGGSGGGGS

SEQ ID NO: 142 - protein, 25 aa, Artificial Sequence
GGGGSGGGGSGGGGSGGGGSGGGGS

SEQ ID NO: 143 - protein, 15 aa, Artificial Sequence
EPKSCDKTHTCPPCP

SEQ ID NO: 144 - protein, 15 aa, Artificial Sequence
EPKSSDKTHTCPPCP

SEQ ID NO: 145 - protein, 15 aa, Artificial Sequence
EPKSSDKTHTPPPPP

SEQ ID NO: 146 - protein, 15 aa, Artificial Sequence
GGGGGDKTHTCPPCP

SEQ ID NO: 147 - protein, 17 aa, Artificial Sequence
EPKSSDKTHTPPPPPRT

SEQ ID NO: 148 - protein, 18 aa, Artificial Sequence
LGGGGSGGGGSGGGGSRT

SEQ ID NO: 149 - protein, 18 aa, Artificial Sequence
LEPKSSDKTHTPPPPPRT

SEQ ID NO: 150 - protein, 19 aa, Artificial Sequence
KLEPKSSDKTHTPPPPPRT

SEQ ID NO: 151 - protein, 19 aa, Artificial Sequence
KLEPKSSDKTHTPPPPPAS

SEQ ID NO: 152 - protein, 9 aa, Artificial Sequence
RTGGGGSKL

SEQ ID NO: 153 - protein, 19 aa, Artificial Sequence
RTGGGGSGGGGSGGGGSKL

SEQ ID NO: 154 - protein, 29 aa, Artificial Sequence
RTGGGGSGGGGSGGGGSGGGGSGGGGSKL

SEQ ID NO: 155 - protein, 6 aa, Artificial Sequence
EPKSSD

SEQ ID NO: 156 - protein, 17 aa, Artificial Sequence
ASGGGGSGGGGSGGGGS

SEQ ID NO: 157 - protein, 2 aa, Artificial Sequence
GS